European Patent Application EP 4 238 984 A1, published September 6, 2023. Title: ANTIBODY-LIKE PROTEIN AND ITS USE. Applicant: CELLEMEDY CO., LTD. The sequence listing filed with the application follows.

SEQUENCE LISTING (30 sequences)

SEQ ID NO: 1 - protein, 183 aa, Homo sapiens
MTTASTSQVRQNYHQDSEAAINRQINLELYASYVYLSMSYYFDRDDVALKNFAKYFLHQSHEEREHAEKLMKLQNQRGGRIFLQDIKKPDCDDWESGLNAMECALHLEKNVNQSLLELHKLATDKNDPHLCDFIETHYLNEQVKAIKELGDHVTNLRKMGAPESGLAEYLFDKHTLGDSDNES

SEQ ID NO: 2 - protein, 12 aa, Homo sapiens
GGSYGSLYAFDI

SEQ ID NO: 3 - protein, 13 aa, Homo sapiens
DLGAGPYYYGKDV

SEQ ID NO: 4 - protein, 6 aa, Homo sapiens
TAQFAY

SEQ ID NO: 5 - protein, 12 aa, Homo sapiens
GYSDYEYNWFDP

SEQ ID NO: 6 - protein, 9 aa, Homo sapiens
VGGAFPMDY

SEQ ID NO: 7 - protein, 19 aa, Homo sapiens
MPSFITLASLSTWEGYFDF

SEQ ID NO: 8 - DNA, 36 bp, Artificial Sequence
  alpha PDL1 F
catatgcaccatcaccatcaccatacgaccgcgtcc

SEQ ID NO: 9 - DNA, 57 bp, Artificial Sequence
  alpha PDL1 R
aagcttctaaatatcaaacgcatacagagaaccataagaaccaccgctttcattatc

SEQ ID NO: 10 - DNA, 36 bp, Artificial Sequence; identical to SEQ ID NO: 8
  alpha PD1 F

SEQ ID NO: 11 - DNA, 60 bp, Artificial Sequence
  alpha PD1 R
aagcttctacacatctttgccatagtaatacgggcccgcgcccagatcgctttcattatc

SEQ ID NO: 12 - DNA, 36 bp, Artificial Sequence; identical to SEQ ID NO: 8
  alpha CTLA4 F

SEQ ID NO: 13 - DNA, 45 bp, Artificial Sequence
  alpha CTLA4 R
aagcttctaatacgcaaactgcgcggtctcgaggctttcattatc

SEQ ID NO: 14 - DNA, 36 bp, Artificial Sequence; identical to SEQ ID NO: 8
  alpha LAG3 F

SEQ ID NO: 15 - DNA, 57 bp, Artificial Sequence
  alpha LAG3 R
aagcttctacggatcaaaccagttatattcataatcgctatagccgctttcattatc

SEQ ID NO: 16 - DNA, 36 bp, Artificial Sequence; identical to SEQ ID NO: 8
  alpha TIM3 F

SEQ ID NO: 17 - DNA, 48 bp, Artificial Sequence
  alpha TIM3 R
aagcttctaataatccatcggaaatgcaccgccaacgctttcattatc

SEQ ID NO: 18 - DNA, 36 bp, Artificial Sequence; identical to SEQ ID NO: 8
  alpha TIGIT F

SEQ ID NO: 19 - DNA, 78 bp, Artificial Sequence
  alpha TIGIT R
aagcttctaaaaatcaaaatagccttcccaggtgctcaggctcgccagggtaataaagctcggcatgctttcattatc

SEQ ID NO: 20 - DNA, 42 bp, Artificial Sequence
  BC alpha PDL1 F
ctgtatgcgtttgatattgaattctgggagagcgggctgaat

SEQ ID NO: 21 - DNA, 51 bp, Artificial Sequence
  BC alpha PDL1 R
agaaccataagaaccaccggatccgtcatcacagtctggtttcttgatatc

SEQ ID NO: 22 - protein, 8 aa, Artificial Sequence
  linker
GGGSGGGT

SEQ ID NO: 23 - protein, 10 aa, Artificial Sequence
  linker
GGGGSGGGGT

SEQ ID NO: 24 - protein, 12 aa, Artificial Sequence
  linker
GGGSGGGTGGGS

SEQ ID NO: 25 - protein, 183 aa, Artificial Sequence
  mutant huHF
MTTASTSQVRQNYHAASEAAINAQINLELYASYVYLSMSYYFDRDDVALKNFAKYFLHQSHEEREHAEKLMKLQNQRGGRIALADIQKPDCDDWESGLNAMECALHLEKNVNQSLLELHKLATDKNDPHLCDFIETHYLNEQVKAIKELGDHVTNLRKMGAPESGLAEYLFDKHTLGDSDNES

SEQ ID NO: 26 - protein, 11 aa, Artificial Sequence
  Her2/neu (herceptin)
WGGDGFYAMDY

SEQ ID NO: 27 - protein, 11 aa, Artificial Sequence
  PD1 (keytruda)
RDYRFDMGFDY

SEQ ID NO: 28 - protein, 7 aa, Artificial Sequence
  PD-L1(tecentriq)
RHWPGGF

SEQ ID NO: 29 - protein, 14 aa, Artificial Sequence
  SARS-Cov
ARGDSSGYYYYFDY

SEQ ID NO: 30 - protein, 11 aa, Artificial Sequence
  CTLA4(yervoy)
ARTGWLGPFDY